European Patent Specification EP 4 092 040 B1, published March 5, 2025. Title: Microorganism That Produces Lysine and Method for Producing Lysine. Applicant: Tianjin Institute of Industrial Biotechnology, Chinese Academy of Sciences. Application EP21741763.3. The sequence listing filed with the application follows.

SEQUENCE LISTING (16 sequences)

SEQ ID NO: 1 - protein, 217 aa, Artificial Sequence
  synthetic
MSIWKRLLVQYPRFADTLTAGQPITLEELATPEVILEAVAKGQEIFGIEQPKHAAQLWFHSLCTAIVGPAVTAMVEFDVIPSLDIRRGQLHNIDGYWFGFRPEEMLVDASLHLSGTQFGESIRVVIDALCAATDLRPAPLWAVASDALGIAASGAGVEAFEEEHAREVAEALIEGMNSVNSVPSPRFNDDDYFIRAGCCMIFHSPRADFCTSCPQKR

SEQ ID NO: 2 - DNA, 654 bp, Artificial Sequence
  synthetic
atgagcatctggaaacgtctgttagtgcagtacccgcgcttcgccgacaccctcacagccggccaacccatcacgctcgaggaattagcaaccccggaagtgatcttggaagctgttgccaaaggccaagaaattttcggcattgagcagccaaaacatgcagcacaactctggtttcactccctgtgcaccgcaattgtcggccccgccgtcaccgccatggtggaattcgatgtcatccccagcctcgacatacgtcgaggtcagctgcataacatcgacggttactggttcggcttcaggccggaggagatgcttgtcgacgcctccctccacctgtcgggcacccaattcggcgagagtatccgcgtggtgattgatgcattatgcgctgccacggatctgcgaccggcacccctgtgggcggttgcctcagatgcgttgggaatcgcagctagcggcgcaggtgtcgaggcctttgaagaagaacatgcccgcgaggtggcggaagccctcattgaaggaatgaatagtgtgaactcagttccatcgccgcggtttaacgacgacgattatttcattcgagctggatgctgcatgattttccactcaccacgagctgatttttgcacgtcgtgcccacagaagaggtga

SEQ ID NO: 3 - DNA, 39 bp, Artificial Sequence
  synthetic
atgacatgattacgaattcacactcctctggctaggtag

SEQ ID NO: 4 - DNA, 21 bp, Artificial Sequence
  synthetic
atgatgtcggtggtgccgtct

SEQ ID NO: 5 - DNA, 38 bp, Artificial Sequence
  synthetic
acggcaccaccgacatcatcttcacctgccctcgttcc

SEQ ID NO: 6 - DNA, 39 bp, Artificial Sequence
  synthetic
ggtcgactctagaggatccacgcaggtgcctgagacctt

SEQ ID NO: 7 - DNA, 39 bp, Artificial Sequence
  synthetic
atgacatgattacgaattcatctctgtgcactcatctac

SEQ ID NO: 8 - DNA, 20 bp, Artificial Sequence
  synthetic
tgctaattcctcgagcgtga

SEQ ID NO: 9 - DNA, 39 bp, Artificial Sequence
  synthetic
cacgctcgaggaattagcacgagctggatgctgcatgat

SEQ ID NO: 10 - DNA, 39 bp, Artificial Sequence
  synthetic
agttattggtgcccttcgattccaaaagtgcagcctaga

SEQ ID NO: 11 - DNA, 24 bp, Artificial Sequence
  synthetic
ttcatgctaattcctcgagcgtga

SEQ ID NO: 12 - DNA, 24 bp, Artificial Sequence
  synthetic
aaactcacgctcgaggaattagca

SEQ ID NO: 13 - DNA, 39 bp, Artificial Sequence
  synthetic
acaggtacagtgtaattcagttttagagctagaaatagc

SEQ ID NO: 14 - DNA, 20 bp, Artificial Sequence
  synthetic
tcagtcacctcctagctgac

SEQ ID NO: 15 - DNA, 20 bp, Artificial Sequence
  synthetic
gtcagctaggaggtgactga

SEQ ID NO: 16 - DNA, 20 bp, Artificial Sequence
  synthetic
tgaattacactgtacctgtt